European Patent Specification EP 3 893 924 B1, published August 21, 2024. Title: ANTIBODIES TO HUMAN COMPLEMENT FACTOR C2b AND METHODS OF USE. Applicant: argenx BVBA Blanchetot, Christophe de Haard, Hans. The sequence listing filed with the application follows.

SEQUENCE LISTING (58 sequences)

SEQ ID NO: 1 - protein, 118 aa, Artificial sequence
  Synthetic polypeptide
  MISC_FEATURE (73)..(75): Any amino acid, provided amino acids 73-75 are not NXS or NXT.
EVQLVQSGAEVKKPGASVKVSCKASGYTFTDYNMDWVRQATGQGLEWIGDINPNYESTGYNQKFKGRATMTVXXXISTAYMELSSLRSEDTAVYYCAREDDHDAFAYWGQGTLVTVSS

SEQ ID NO: 2 - protein, 111 aa, Artificial sequence
  Synthetic polypeptide
DNVLTQSPDSLAVSLGERATISCRASKSVRTSGYNYMHWYQQKPGQPPKLLIYLASNLKSGVPDRFSGSGSGTDFTLTISSLQAEDAATYYCQHSRELPYTFGQGTKLEIK

SEQ ID NO: 3 - protein, 118 aa, Artificial sequence
  Synthetic polypeptide
EVQLVQSGAEVKKPGASVKVSCKASGYTFTDYNMDWVRQATGQGLEWIGDINPNYESTGYNQKFKGRATMTVDKSISTAYMELSSLRSEDTAVYYCAREDDHDAFAYWGQGTLVTVSS

SEQ ID NO: 4 - protein, 329 aa, Artificial sequence
  Synthetic polypeptide
ASTKGPSVFPLAPSSKSTSGGTAALGCLVKDYFPEPVTVSWNSGALTSGVHTFPAVLQSSGLYSLSSVVTVPSSSLGTQTYICNVNHKPSNTKVDKKVEPKSCDKTHTCPPCPAPEAAGGPSVFLFPPKPKDTLMISRTPEVTCVVVDVSHEDPEVKFNWYVDGVEVHNAKTKPREEQYNSTYRVVSVLTVLHQDWLNGKEYKCKVSNKALPAPIEKTISKAKGQPREPQVYTLPPSRDELTKNQVSLTCLVKGFYPSDIAVEWESNGQPENNYKTTPPVLDSDGSFFLYSKLTVDKSRWQQGNVFSCSVMHEALKFHYTQKSLSLSPG

SEQ ID NO: 5 - protein, 327 aa, Artificial sequence
  Synthetic polypeptide
ASTKGPSVFPLAPCSRSTSESTAALGCLVKDYFPEPVTVSWNSGALTSGVHTFPAVLQSSGLYSLSSVVTVPSSSLGTKTYTCNVDHKPSNTKVDKRVESKYGPPCPPCPAPEFLGGPSVFLFPPKPKDTLMISRTPEVTCVVVDVSQEDPEVQFNWYVDGVEVHNAKTKPREEQFNSTYRVVSVLTVLHQDWLNGKEYKCKVSNKGLPSSIEKTISKAKGQPREPQVYTLPPSQEEMTKNQVSLTCLVKGFYPSDIAVEWESNGQPENNYKTTPPVLDSDGSFFLYSRLTVDKSRWQEGNVFSCSVMHEALKFHYTQKSLSLSPGK

SEQ ID NO: 6 - protein, 447 aa, Artificial sequence
  Synthetic polypeptide
EVQLVQSGAEVKKPGASVKVSCKASGYTFTDYNMDWVRQATGQGLEWIGDINPNYESTGYNQKFKGRATMTVDKSISTAYMELSSLRSEDTAVYYCAREDDHDAFAYWGQGTLVTVSSASTKGPSVFPLAPSSKSTSGGTAALGCLVKDYFPEPVTVSWNSGALTSGVHTFPAVLQSSGLYSLSSVVTVPSSSLGTQTYICNVNHKPSNTKVDKKVEPKSCDKTHTCPPCPAPEAAGGPSVFLFPPKPKDTLMISRTPEVTCVVVDVSHEDPEVKFNWYVDGVEVHNAKTKPREEQYNSTYRVVSVLTVLHQDWLNGKEYKCKVSNKALPAPIEKTISKAKGQPREPQVYTLPPSRDELTKNQVSLTCLVKGFYPSDIAVEWESNGQPENNYKTTPPVLDSDGSFFLYSKLTVDKSRWQQGNVFSCSVMHEALKFHYTQKSLSLSPG

SEQ ID NO: 7 - protein, 218 aa, Artificial sequence
  Synthetic polypeptide
DNVLTQSPDSLAVSLGERATISCRASKSVRTSGYNYMHWYQQKPGQPPKLLIYLASNLKSGVPDRFSGSGSGTDFTLTISSLQAEDAATYYCQHSRELPYTFGQGTKLEIKRTVAAPSVFIFPPSDEQLKSGTASVVCLLNNFYPREAKVQWKVDNALQSGNSQESVTEQDSKDSTYSLSSTLTLSKADYEKHKVYACEVTHQGLSSPVTKSFNRGEC

SEQ ID NO: 8 - protein, 445 aa, Artificial sequence
  Synthetic polypeptide
EVQLVQSGAEVKKPGASVKVSCKASGYTFTDYNMDWVRQATGQGLEWIGDINPNYESTGYNQKFKGRATMTVDKSISTAYMELSSLRSEDTAVYYCAREDDHDAFAYWGQGTLVTVSSASTKGPSVFPLAPCSRSTSESTAALGCLVKDYFPEPVTVSWNSGALTSGVHTFPAVLQSSGLYSLSSVVTVPSSSLGTKTYTCNVDHKPSNTKVDKRVESKYGPPCPPCPAPEFLGGPSVFLFPPKPKDTLMISRTPEVTCVVVDVSQEDPEVQFNWYVDGVEVHNAKTKPREEQFNSTYRVVSVLTVLHQDWLNGKEYKCKVSNKGLPSSIEKTISKAKGQPREPQVYTLPPSQEEMTKNQVSLTCLVKGFYPSDIAVEWESNGQPENNYKTTPPVLDSDGSFFLYSRLTVDKSRWQEGNVFSCSVMHEALKFHYTQKSLSLSPGK

SEQ ID NO: 9 - protein, 10 aa, Homo sapiens
EPKSCDKTHT

SEQ ID NO: 10 - protein, 5 aa, Homo sapiens
CPPCP

SEQ ID NO: 11 - protein, 8 aa, Homo sapiens
APELLGGP

SEQ ID NO: 12 - protein, 3 aa, Homo sapiens
ERK

SEQ ID NO: 13 - protein, 10 aa, Homo sapiens
CCVECPPPCP

SEQ ID NO: 14 - protein, 7 aa, Homo sapiens
APPVAGP

SEQ ID NO: 15 - protein, 12 aa, Homo sapiens
ELKTPLGDTTHT

SEQ ID NO: 16 - protein, 50 aa, Homo sapiens
CPRCPEPKSCDTPPPCPRCPEPKSCDTPPPCPRCPEPKSCDTPPPCPRCP

SEQ ID NO: 17 - protein, 8 aa, Homo sapiens
APELLGGP

SEQ ID NO: 18 - protein, 7 aa, Homo sapiens
ESKYGPP

SEQ ID NO: 19 - protein, 5 aa, Homo sapiens
CPSCP

SEQ ID NO: 20 - protein, 8 aa, Homo sapiens
APEFLGGP

SEQ ID NO: 21 - protein, 752 aa, Homo sapiens
MGPLMVLFCLLFLYPGLADSAPSCPQNVNISGGTFTLSHGWAPGSLLTYSCPQGLYPSPASRLCKSSGQWQTPGATRSLSKAVCKPVRCPAPVSFENGIYTPRLGSYPVGGNVSFECEDGFILRGSPVRQCRPNGMWDGETAVCDNGAGHCPNPGISLGAVRTGFRFGHGDKVRYRCSSNLVLTGSSERECQGNGVWSGTEPICRQPYSYDFPEDVAPALGTSFSHMLGATNPTQKTKESLGRKIQIQRSGHLNLYLLLDCSQSVSENDFLIFKESASLMVDRIFSFEINVSVAIITFASEPKVLMSVLNDNSRDMTEVISSLENANYKDHENGTGTNTYAALNSVYLMMNNQMRLLGMETMAWQEIRHAIILLTDGKSNMGGSPKTAVDHIREILNINQKRNDYLDIYAIGVGKLDVDWRELNELGSKKDGERHAFILQDTKALHQVFEHMLDVSKLTDTICGVGNMSANASDQERTPWHVTIKPKSQETCRGALISDQWVLTAAHCFRDGNDHSLWRVNVGDPKSQWGKEFLIEKAVISPGFDVFAKKNQGILEFYGDDIALLKLAQKVKMSTHARPICLPCTMEANLALRRPQGSTCRDHENELLNKQSVPAHFVALNGSKLNINLKMGVEWTSCAEVVSQEKTMFPNLTDVREVVTDQFLCSGTQEDESPCKGESGGAVFLERRFRFFQVGLVSWGLYNPCLGSADKNSRKRAPRSKVPPPRDFHINLFRMQPWLRQHLGDVLNFLPL

SEQ ID NO: 22 - protein, 5 aa, Artificial sequence
  Synthetic peptide
DYNMD

SEQ ID NO: 23 - protein, 17 aa, Artificial sequence
  Synthetic peptide
DINPNYESTGYNQKFKG

SEQ ID NO: 24 - protein, 9 aa, Artificial sequence
  Synthetic peptide
EDDHDAFAY

SEQ ID NO: 25 - protein, 15 aa, Artificial sequence
  Synthetic peptide
RASKSVRTSGYNYMH

SEQ ID NO: 26 - protein, 7 aa, Artificial sequence
  Synthetic peptide
LASNLKS

SEQ ID NO: 27 - protein, 9 aa, Artificial sequence
  Synthetic peptide
QHSRELPYT

SEQ ID NO: 28 - protein, 118 aa, Artificial sequence
  Synthetic polypeptide
EVQLVQSGAEVKKPGASVKVSCKASGYTFTDYNMDWVRQATGQGLEWIGDINPNYESTGYNQKFKGRATMTVNKSISTAYMELSSLRSEDTAVYYCAREDDHDAFAYWGQGTLVTVSS

SEQ ID NO: 29 - protein, 330 aa, Artificial sequence [sequence omitted]

SEQ ID NO: 30 - protein, 327 aa, Artificial sequence
  Synthetic polypeptide
ASTKGPSVFPLAPCSRSTSESTAALGCLVKDYFPEPVTVSWNSGALTSGVHTFPAVLQSSGLYSLSSVVTVPSSSLGTKTYTCNVDHKPSNTKVDKRVESKYGPPCPSCPAPEFLGGPSVFLFPPKPKDTLMISRTPEVTCVVVDVSQEDPEVQFNWYVDGVEVHNAKTKPREEQFNSTYRVVSVLTVLHQDWLNGKEYKCKVSNKGLPSSIEKTISKAKGQPREPQVYTLPPSQEEMTKNQVSLTCLVKGFYPSDIAVEWESNGQPENNYKTTPPVLDSDGSFFLYSRLTVDKSRWQEGNVFSCSVMHEALHNHYTQKSLSLSLGK

SEQ ID NO: 31 - protein, 327 aa, Artificial sequence
  Synthetic polypeptide
ASTKGPSVFPLAPCSRSTSESTAALGCLVKDYFPEPVTVSWNSGALTSGVHTFPAVLQSSGLYSLSSVVTVPSSSLGTKTYTCNVDHKPSNTKVDKRVESKYGPPCPPCPAPEFLGGPSVFLFPPKPKDTLMISRTPEVTCVVVDVSQEDPEVQFNWYVDGVEVHNAKTKPREEQFNSTYRVVSVLTVLHQDWLNGKEYKCKVSNKGLPSSIEKTISKAKGQPREPQVYTLPPSQEEMTKNQVSLTCLVKGFYPSDIAVEWESNGQPENNYKTTPPVLDSDGSFFLYSRLTVDKSRWQEGNVFSCSVMHEALHNHYTQKSLSLSPGK

SEQ ID NO: 32 - protein, 448 aa, Artificial sequence
  Synthetic polypeptide
EVQLVQSGAEVKKPGASVKVSCKASGYTFTDYNMDWVRQATGQGLEWIGDINPNYESTGYNQKFKGRATMTVDKSISTAYMELSSLRSEDTAVYYCAREDDHDAFAYWGQGTLVTVSSASTKGPSVFPLAPSSKSTSGGTAALGCLVKDYFPEPVTVSWNSGALTSGVHTFPAVLQSSGLYSLSSVVTVPSSSLGTQTYICNVNHKPSNTKVDKKVEPKSCDKTHTCPPCPAPELLGGPSVFLFPPKPKDTLMISRTPEVTCVVVDVSHEDPEVKFNWYVDGVEVHNAKTKPREEQYNSTYRVVSVLTVLHQDWLNGKEYKCKVSNKALPAPIEKTISKAKGQPREPQVYTLPPSRDELTKNQVSLTCLVKGFYPSDIAVEWESNGQPENNYKTTPPVLDSDGSFFLYSKLTVDKSRWQQGNVFSCSVMHEALHNHYTQKSLSLSPGK

SEQ ID NO: 33 - protein, 445 aa, Artificial sequence
  Synthetic polypeptide
EVQLVQSGAEVKKPGASVKVSCKASGYTFTDYNMDWVRQATGQGLEWIGDINPNYESTGYNQKFKGRATMTVDKSISTAYMELSSLRSEDTAVYYCAREDDHDAFAYWGQGTLVTVSSASTKGPSVFPLAPCSRSTSESTAALGCLVKDYFPEPVTVSWNSGALTSGVHTFPAVLQSSGLYSLSSVVTVPSSSLGTKTYTCNVDHKPSNTKVDKRVESKYGPPCPSCPAPEFLGGPSVFLFPPKPKDTLMISRTPEVTCVVVDVSQEDPEVQFNWYVDGVEVHNAKTKPREEQFNSTYRVVSVLTVLHQDWLNGKEYKCKVSNKGLPSSIEKTISKAKGQPREPQVYTLPPSQEEMTKNQVSLTCLVKGFYPSDIAVEWESNGQPENNYKTTPPVLDSDGSFFLYSRLTVDKSRWQEGNVFSCSVMHEALHNHYTQKSLSLSLGK

SEQ ID NO: 34 - protein, 445 aa, Artificial sequence
  Synthetic polypeptide
EVQLVQSGAEVKKPGASVKVSCKASGYTFTDYNMDWVRQATGQGLEWIGDINPNYESTGYNQKFKGRATMTVDKSISTAYMELSSLRSEDTAVYYCAREDDHDAFAYWGQGTLVTVSSASTKGPSVFPLAPCSRSTSESTAALGCLVKDYFPEPVTVSWNSGALTSGVHTFPAVLQSSGLYSLSSVVTVPSSSLGTKTYTCNVDHKPSNTKVDKRVESKYGPPCPPCPAPEFLGGPSVFLFPPKPKDTLMISRTPEVTCVVVDVSQEDPEVQFNWYVDGVEVHNAKTKPREEQFNSTYRVVSVLTVLHQDWLNGKEYKCKVSNKGLPSSIEKTISKAKGQPREPQVYTLPPSQEEMTKNQVSLTCLVKGFYPSDIAVEWESNGQPENNYKTTPPVLDSDGSFFLYSRLTVDKSRWQEGNVFSCSVMHEALHNHYTQKSLSLSPGK

SEQ ID NO: 35 - DNA, 354 bp, Artificial sequence
  Synthetic polynucleottide
gaagtgcagctggtgcagtctggcgccgaagtgaagaaacctggcgcctccgtgaaggtgtcctgcaaggcttccggctacacctttaccgactacaacatggactgggtgcgacaggctaccggccagggcctggaatggatcggcgacatcaaccccaactacgagtccaccggctacaaccagaagttcaagggcagagccaccatgaccgtggacaagtccatctccaccgcctacatggaactgtcctccctgcggagcgaggacaccgccgtgtactactgcgccagagaggacgaccacgacgcctttgcttattggggccagggcaccctcgtgaccgtgtcctct

SEQ ID NO: 36 - DNA, 333 bp, Artificial sequence
  Synthetic polynucleottide
gacaacgtgctgacccagtcccctgactccctggctgtgtctctgggcgagagagccaccatctcttgccgggcctctaagtccgtgcggacctccggctacaactacatgcactggtatcagcagaagcccggccagccccccaagctgctgatctacctggcctccaacctgaagtccggcgtgcccgacagattctccggctctggctctggcaccgactttaccctgaccatcagctccctgcaggccgaggatgccgccacctactactgccagcactccagagagctgccctacacctttggccagggcaccaagctggaaatcaag

SEQ ID NO: 37 - DNA, 1344 bp, Artificial sequence
  Synthetic polypeptide
gaagttcagctggttcagtctggcgccgaagtgaagaaacctggcgcctctgtgaaggtgtcctgcaaggcttctggctacacctttaccgactacaacatggactgggtccgacaggctaccggacagggacttgagtggatcggcgacatcaaccccaactacgagtccaccggctacaaccagaagttcaagggcagagccaccatgaccgtggacaagtccatctccaccgcctacatggaactgtccagcctgagatctgaggacaccgccgtgtactactgcgccagagaggatgatcacgacgcctttgcttattggggccagggcacactggtcaccgtgtcctctgccagtacaaaaggtccaagtgtgttccctcttgctccctcatccaagagtaccagtggaggcaccgccgctcttggctgcttggttaaggattatttcccagagcctgtcactgtttcatggaactccggcgccttgacatctggtgtgcatacctttccagccgtgctgcagtcaagtggcctctacagcctcagtagcgtggtcactgtgcccagcagctctctcggcacacaaacttatatctgtaatgtgaatcataagccttcaaataccaaggtggataagaaagtggaaccaaaatcatgtgacaagacacacacctgccctccttgtccagcccccgaactgctgggtgggcccagcgtgttcctgtttcctcctaaacccaaagacactctgatgattagtaggaccccagaagtcacttgcgtggtggttgacgtgtcacatgaagatcccgaggtcaagttcaattggtatgttgacggggtcgaagttcacaacgctaaaactaaaccaagagaggaacagtataactctacctaccgggtggtgagtgttctgactgtcctccatcaagactggctgaatggcaaagaatacaagtgtaaggtgagcaacaaagccctgcccgctcctatagagaaaacaatatccaaagccaaaggtcaacctcgcgagccacaggtgtacaccctcccaccaagccgcgatgaacttactaagaaccaagtctctcttacttgcctggttaaggggttctatccatccgacattgcagtcgagtgggagtctaatggacagcctgagaacaactacaaaaccacccctcctgttctggattctgacggatctttcttcctttattctaaactcaccgtggataaaagcaggtggcagcagggcaacgtgttcagctgttccgttatgcatgaggccctgcataaccattatacccagaagtctttgtccctcagtccaggaaag

SEQ ID NO: 38 - DNA, 1341 bp, Artificial sequence
  Synthetic polynucleottide
gaagttcagctggttcagtctggcgccgaagtgaagaaacctggcgcctctgtgaaggtgtcctgcaaggcttctggctacacctttaccgactacaacatggactgggtccgacaggctaccggacagggacttgagtggatcggcgacatcaaccccaactacgagtccaccggctacaaccagaagttcaagggcagagccaccatgaccgtggacaagtccatctccaccgcctacatggaactgtccagcctgagatctgaggacaccgccgtgtactactgcgccagagaggatgatcacgacgcctttgcttattggggccagggcacactggtcaccgtgtcctctgcttctaccaagggacccagcgtgttccctctggctccttccagcaagtctacctctggcggaacagctgctctgggctgcctggtcaaggactactttcctgagcctgtgaccgtgtcttggaactctggcgctctgacatctggcgtgcacacctttccagctgtgctgcagtcctccggcctgtactctctgtcctctgtcgtgaccgtgccttccagctctctgggaacccagacctacatctgcaatgtgaaccacaagccttccaacaccaaggtggacaagaaggtggaacccaagtcctgcgacaagacccacacctgtcctccatgtcctgctccagaagctgctggcggcccttccgtgtttctgttccctccaaagcctaaggacaccctgatgatctctcggacccctgaagtgacctgcgtggtggtggatgtgtctcacgaggacccagaagtgaagttcaattggtacgtggacggcgtggaagtgcacaacgccaagaccaagcctagagaggaacagtacaactccacctacagagtggtgtccgtgctgaccgtgctgcaccaggattggctgaacggcaaagagtacaagtgcaaggtgtccaacaaggccctgcctgctcctatcgaaaagaccatctccaaggccaagggccagcctagggaaccccaggtttacaccttgcctccatctcgggacgagctgaccaagaaccaggtgtccctgacctgtctcgtgaagggcttctacccctccgatatcgccgtggaatgggagtctaatggccagccagagaacaactacaagacaacccctcctgtgctggactccgacggctcattctttctgtactccaagctgacagtggataagtcccggtggcagcagggcaacgtgttctcctgttctgtgatgcacgaggccctgaagttccactacacacagaagtctctgtctctgagccccggc

SEQ ID NO: 39 - DNA, 1335 bp, Artificial sequence
  Synthetic polypeptide
gaagtgcagctggtgcagtctggcgccgaagtgaagaaacctggcgcctccgtgaaggtgtcctgcaaggcttccggctacacctttaccgactacaacatggactgggtgcgacaggctaccggccagggcctggaatggatcggcgacatcaaccccaactacgagtccaccggctacaaccagaagttcaagggcagagccaccatgaccgtggacaagtccatctccaccgcctacatggaactgtcctccctgcggagcgaggacaccgccgtgtactactgcgccagagaggacgaccacgacgcctttgcttattggggccagggcaccctcgtgaccgtgtcctctgcttctaccaagggcccctccgtgttccctctggccccttgctccagatccacctccgagtctaccgccgctctgggctgcctcgtgaaggactacttccccgagcccgtgacagtgtcttggaactctggcgccctgacctccggcgtgcacacctttccagctgtgctgcagtcctccggcctgtactccctgtcctccgtcgtgactgtgccctccagctctctgggcaccaagacctacacctgtaacgtggaccacaagccctccaacaccaaggtggacaagcgggtggaatctaagtacggccctccctgccctccttgcccagcccctgaatttctgggcggacccagcgtgttcctgttccccccaaagcccaaggacaccctgatgatctcccggacccccgaagtgacctgcgtggtggtggatgtgtcccaggaagatcccgaggtgcagttcaattggtacgtggacggcgtggaagtgcacaacgccaagaccaagcctagagaggaacagttcaactccacctaccgggtggtgtccgtgctgaccgtgctgcaccaggattggctgaacggcaaagagtacaagtgcaaggtgtccaacaagggcctgccttccagcatcgaaaagaccatctccaaggccaagggccagccccgggaaccccaggtgtacacactgcctccaagccaggaagagatgaccaagaaccaggtgtccctgacctgtctcgtgaaaggcttctacccctccgatatcgccgtggaatgggagtccaacggccagcctgagaacaactacaagaccaccccccctgtgctggactccgacggctccttcttcctgtactctcgcctgaccgtggataagtcccggtggcaggaaggcaacgtgttctcctgctccgtgatgcacgaggccctgcacaaccactatacccagaagtccctgtccctgtctctgggaaag

SEQ ID NO: 40 - DNA, 1349 bp, Artificial sequence
  Synthetic polypeptide
gaagtgcagctggtgcagtctggcgccgaagtgaaaaaacctggcgcctccgtgaaggtgtcctgcaaggctagcggctacacctttaccgactacaacatggactgggtccgacaggccacaggacagggactcgagtggatcggcgacatcaaccccaactacgagagcaccggctacaaccagaagttcaagggcagagccaccatgaccgtggacaagagcatcagcaccgcctacatggaactgagcagcctgagaagcgaggacaccgccgtgtactactgcgccagagaggatgatcacgacgcctttgcctattggggccagggcacactggtcaccgttagctctgctagcaccaagggcccatcggtcttccccctggcgccctgctccaggagcacctccgagagcacagccgccctgggctgcctggtcaaggactacttccccgaaccggtgacggtgtcgtggaactcaggcgccctgaccagcggcgtgcacaccttcccggctgtcctacagtcctcaggactctactccctcagcagcgtggtgaccgtgccctccagcagcttgggcacgaagacctacacctgcaacgtagatcacaagcccagcaacaccaaggtggacaagagagttgagtccaaatatggtcccccatgcccaccatgcccagcacctgagttcctggggggaccatcagtcttcctgttccccccaaaacccaaggacactctcatgatctcccggacccctgaggtcacgtgcgtggtggtggacgtgagccaggaagaccccgaggtccagttcaactggtacgtggatggcgtggaggtgcataatgccaagacaaagccgcgggaggagcagttcaacagcacgtaccgtgtggtcagcgtcctcaccgtcctgcaccaggactggctgaacggcaaggagtacaagtgcaaggtctccaacaaaggcctcccgtcctccatcgagaaaaccatctccaaagccaaagggcagccccgagagccacaggtgtacaccctgcccccatcccaggaggagatgaccaagaaccaggtcagcctgacctgcctggtcaaaggcttctaccccagcgacatcgccgtggagtgggagagcaatgggcagccggagaacaactacaagaccacgcctcccgtgctggactccgacggctccttcttcctctacagcaggctcaccgtggacaagagcaggtggcaggaggggaatgtcttctcatgctccgtgatgcatgaggctctgcacaaccactacacacagaagagcctctccctgtctccgggtaaatgagtcctagctgg

SEQ ID NO: 41 - DNA, 1335 bp, Artificial sequence
  Synthetic polynucleottide
gaagtgcagctggtgcagtctggcgccgaagtgaaaaaacctggcgcctccgtgaaggtgtcctgcaaggctagcggctacacctttaccgactacaacatggactgggtccgacaggccacaggacagggactcgagtggatcggcgacatcaaccccaactacgagagcaccggctacaaccagaagttcaagggcagagccaccatgaccgtggacaagagcatcagcaccgcctacatggaactgagcagcctgagaagcgaggacaccgccgtgtactactgcgccagagaggatgatcacgacgcctttgcctattggggccagggcacactggtcaccgttagctctgctagcaccaagggcccatcggtcttccccctggcgccctgctccaggagcacctccgagagcacagccgccctgggctgcctggtcaaggactacttccccgaaccggtgacggtgtcgtggaactcaggcgccctgaccagcggcgtgcacaccttcccggctgtcctacagtcctcaggactctactccctcagcagcgtggtgaccgtgccctccagcagcttgggcacgaagacctacacctgcaacgtagatcacaagcccagcaacaccaaggtggacaagagagttgagtccaaatatggtcccccatgcccaccatgcccagcacctgagttcctggggggaccatcagtcttcctgttccccccaaaacccaaggacactctcatgatctcccggacccctgaggtcacgtgcgtggtggtggacgtgagccaggaagaccccgaggtccagttcaactggtacgtggatggcgtggaggtgcataatgccaagacaaagccgcgggaggagcagttcaacagcacgtaccgtgtggtcagcgtcctcaccgtcctgcaccaggactggctgaacggcaaggagtacaagtgcaaggtctccaacaaaggcctcccgtcctccatcgagaaaaccatctccaaagccaaagggcagccccgagagccacaggtgtacaccctgcccccatcccaggaggagatgaccaagaaccaggtcagcctgacctgcctggtcaaaggcttctaccccagcgacatcgccgtggagtgggagagcaatgggcagccggagaacaactacaagaccacgcctcccgtgctggactccgacggctccttcttcctctacagcaggctcaccgtggacaagagcaggtggcaggaggggaatgtcttctcatgctccgtgatgcatgaggctctgaagttccactacacacagaagagcctctccctgtctccgggtaaa

SEQ ID NO: 42 - DNA, 654 bp, Artificial sequence
  Synthetic polypeptide
gacaacgtgctgacccagtcccctgactccctggctgtgtctctgggcgagagagccaccatctcttgccgggcctctaagtccgtgcggacctccggctacaactacatgcactggtatcagcagaagcccggccagccccccaagctgctgatctacctggcctccaacctgaagtccggcgtgcccgacagattctccggctctggctctggcaccgactttaccctgaccatcagctccctgcaggccgaggatgccgccacctactactgccagcactccagagagctgccctacacctttggccagggcaccaagctggaaatcaagcggaccgtggccgctccctccgtgttcatcttcccaccttccgacgagcagctgaagtctggcacagcctccgtcgtgtgcctgctgaacaacttctacccccgcgaggccaaggtgcagtggaaggtggacaacgccctgcagtccggcaactcccaggaatccgtgaccgagcaggactccaaggacagcacctactccctgtcctccaccctgaccctgtccaaggccgactacgagaagcacaaggtgtacgcctgcgaagtgacccaccagggcctgtctagccccgtgaccaagtctttcaaccggggcgagtgc

SEQ ID NO: 43 - protein, 509 aa, Homo sapiens
KIQIQRSGHLNLYLLLDCSQSVSENDFLIFKESASLMVDRIFSFEINVSVAIITFASEPKVLMSVLNDNSRDMTEVISSLENANYKDHENGTGTNTYAALNSVYLMMNNQMRLLGMETMAWQEIRHAIILLTDGKSNMGGSPKTAVDHIREILNINQKRNDYLDIYAIGVGKLDVDWRELNELGSKKDGERHAFILQDTKALHQVFEHMLDVSKLTDTICGVGNMSANASDQERTPWHVTIKPKSQETCRGALISDQWVLTAAHCFRDGNDHSLWRVNVGDPKSQWGKEFLIEKAVISPGFDVFAKKNQGILEFYGDDIALLKLAQKVKMSTHARPICLPCTMEANLALRRPQGSTCRDHENELLNKQSVPAHFVALNGSKLNINLKMGVEWTSCAEVVSQEKTMFPNLTDVREVVTDQFLCSGTQEDESPCKGESGGAVFLERRFRFFQVGLVSWGLYNPCLGSADKNSRKRAPRSKVPPPRDFHINLFRMQPWLRQHLGDVLNFLPL

SEQ ID NO: 44 - protein, 223 aa, Homo sapiens
APSCPQNVNISGGTFTLSHGWAPGSLLTYSCPQGLYPSPASRLCKSSGQWQTPGATRSLSKAVCKPVRCPAPVSFENGIYTPRLGSYPVGGNVSFECEDGFILRGSPVRQCRPNGMWDGETAVCDNGAGHCPNPGISLGAVRTGFRFGHGDKVRYRCSSNLVLTGSSERECQGNGVWSGTEPICRQPYSYDFPEDVAPALGTSFSHMLGATNPTQKTKESLGR

SEQ ID NO: 45 - protein, 65 aa, Homo sapiens
PSCPQNVNISGGTFTLSHGWAPGSLLTYSCPQGLYPSPASRLCKSSGQWQTPGATRSLSKAVCKP

SEQ ID NO: 46 - protein, 61 aa, Homo sapiens
VRCPAPVSFENGIYTPRLGSYPVGGNVSFECEDGFILRGSPVRQCRPNGMWDGETAVCDNG

SEQ ID NO: 47 - protein, 58 aa, Homo sapiens
GHCPNPGISLGAVRTGFRFGHGDKVRYRCSSNLVLTGSSERECQGNGVWSGTEPICRQ

SEQ ID NO: 48 - protein, 199 aa, Homo sapiens
NLYLLLDCSQSVSENDFLIFKESASLMVDRIFSFEINVSVAIITFASEPKVLMSVLNDNSRDMTEVISSLENANYKDHENGTGTNTYAALNSVYLMMNNQMRLLGMETMAWQEIRHAIILLTDGKSNMGGSPKTAVDHIREILNINQKRNDYLDIYAIGVGKLDVDWRELNELGSKKDGERHAFILQDTKALHQVFEHM

SEQ ID NO: 49 - protein, 281 aa, Homo sapiens
GVGNMSANASDQERTPWHVTIKPKSQETCRGALISDQWVLTAAHCFRDGNDHSLWRVNVGDPKSQWGKEFLIEKAVISPGFDVFAKKNQGILEFYGDDIALLKLAQKVKMSTHARPICLPCTMEANLALRRPQGSTCRDHENELLNKQSVPAHFVALNGSKLNINLKMGVEWTSCAEVVSQEKTMFPNLTDVREVVTDQFLCSGTQEDESPCKGESGGAVFLERRFRFFQVGLVSWGLYNPCLGSADKNSRKRAPRSKVPPPRDFHINLFRMQPWLRQHLG

SEQ ID NO: 50 - protein, 764 aa, Homo sapiens
MGSNLSPQLCLMPFILGLLSGGVTTTPWSLARPQGSCSLEGVEIKGGSFRLLQEGQALEYVCPSGFYPYPVQTRTCRSTGSWSTLKTQDQKTVRKAECRAIHCPRPHDFENGEYWPRSPYYNVSDEISFHCYDGYTLRGSANRTCQVNGRWSGQTAICDNGAGYCSNPGIPIGTRKVGSQYRLEDSVTYHCSRGLTLRGSQRRTCQEGGSWSGTEPSCQDSFMYDTPQEVAEAFLSSLTETIEGVDAEDGHGPGEQQKRKIVLDPSGSMNIYLVLDGSDSIGASNFTGAKKCLVNLIEKVASYGVKPRYGLVTYATYPKIWVKVSEADSSNADWVTKQLNEINYEDHKLKSGTNTKKALQAVYSMMSWPDDVPPEGWNRTRHVIILMTDGLHNMGGDPITVIDEIRDLLYIGKDRKNPREDYLDVYVFGVGPLVNQVNINALASKKDNEQHVFKVKDMENLEDVFYQMIDESQSLSLCGMVWEHRKGTDYHKQPWQAKISVIRPSKGHESCMGAVVSEYFVLTAAHCFTVDDKEHSIKVSVGGEKRDLEIEVVLFHPNYNINGKKEAGIPEFYDYDVALIKLKNKLKYGQTIRPICLPCTEGTTRALRLPPTTTCQQQKEELLPAQDIKALFVSEEEKKLTRKEVYIKNGDKKGSCERDAQYAPGYDKVKDISEVVTPRFLCTGGVSPYADPNTCRGDSGGPLIVHKRSRFIQVGVISWGVVDVCKNQKRQKQVPAHARDFHINLFQVLPWLKEKLQDEDLGFL

SEQ ID NO: 51 - protein, 234 aa, Homo sapiens
TPWSLARPQGSCSLEGVEIKGGSFRLLQEGQALEYVCPSGFYPYPVQTRTCRSTGSWSTLKTQDQKTVRKAECRAIHCPRPHDFENGEYWPRSPYYNVSDEISFHCYDGYTLRGSANRTCQVNGRWSGQTAICDNGAGYCSNPGIPIGTRKVGSQYRLEDSVTYHCSRGLTLRGSQRRTCQEGGSWSGTEPSCQDSFMYDTPQEVAEAFLSSLTETIEGVDAEDGHGPGEQQKR

SEQ ID NO: 52 - protein, 505 aa, Homo sapiens
KIVLDPSGSMNIYLVLDGSDSIGASNFTGAKKCLVNLIEKVASYGVKPRYGLVTYATYPKIWVKVSEADSSNADWVTKQLNEINYEDHKLKSGTNTKKALQAVYSMMSWPDDVPPEGWNRTRHVIILMTDGLHNMGGDPITVIDEIRDLLYIGKDRKNPREDYLDVYVFGVGPLVNQVNINALASKKDNEQHVFKVKDMENLEDVFYQMIDESQSLSLCGMVWEHRKGTDYHKQPWQAKISVIRPSKGHESCMGAVVSEYFVLTAAHCFTVDDKEHSIKVSVGGEKRDLEIEVVLFHPNYNINGKKEAGIPEFYDYDVALIKLKNKLKYGQTIRPICLPCTEGTTRALRLPPTTTCQQQKEELLPAQDIKALFVSEEEKKLTRKEVYIKNGDKKGSCERDAQYAPGYDKVKDISEVVTPRFLCTGGVSPYADPNTCRGDSGGPLIVHKRSRFIQVGVISWGVVDVCKNQKRQKQVPAHARDFHINLFQVLPWLKEKLQDEDLGFL

SEQ ID NO: 53 - protein, 66 aa, Homo sapiens
GSCSLEGVEIKGGSFRLLQEGQALEYVCPSGFYPYPVQTRTCRSTGSWSTLKTQDQKTVRKAECRA

SEQ ID NO: 54 - protein, 60 aa, Homo sapiens
IHCPRPHDFENGEYWPRSPYYNVSDEISFHCYDGYTLRGSANRTCQVNGRWSGQTAICDN

SEQ ID NO: 55 - protein, 58 aa, Homo sapiens
GYCSNPGIPIGTRKVGSQYRLEDSVTYHCSRGLTLRGSQRRTCQEGGSWSGTEPSCQD

SEQ ID NO: 56 - protein, 200 aa, Homo sapiens
NIYLVLDGSDSIGASNFTGAKKCLVNLIEKVASYGVKPRYGLVTYATYPKIWVKVSEADSSNADWVTKQLNEINYEDHKLKSGTNTKKALQAVYSMMSWPDDVPPEGWNRTRHVIILMTDGLHNMGGDPITVIDEIRDLLYIGKDRKNPREDYLDVYVFGVGPLVNQVNINALASKKDNEQHVFKVKDMENLEDVFYQMI

SEQ ID NO: 57 - protein, 281 aa, Homo sapiens
LCGMVWEHRKGTDYHKQPWQAKISVIRPSKGHESCMGAVVSEYFVLTAAHCFTVDDKEHSIKVSVGGEKRDLEIEVVLFHPNYNINGKKEAGIPEFYDYDVALIKLKNKLKYGQTIRPICLPCTEGTTRALRLPPTTTCQQQKEELLPAQDIKALFVSEEEKKLTRKEVYIKNGDKKGSCERDAQYAPGYDKVKDISEVVTPRFLCTGGVSPYADPNTCRGDSGGPLIVHKRSRFIQVGVISWGVVDVCKNQKRQKQVPAHARDFHINLFQVLPWLKEKLQ

SEQ ID NO: 58 - protein, 61 aa, Mus musculus
VRCLAPSSFENGIYFPRLVSYPVGSNVSFECEQDFTLRGSPVRYCRPNGLWDGETAVCDNG